European Patent Specification EP 3 551 749 B1, published September 27, 2023. Title: COMPOSITIONS AND METHODS FOR IN VITRO CULTIVATION AND/OR EXPANSION OF REGULATORY T CELLS. Applicant: East Carolina University Wilkinson, Daniel Stephen Mannie, Mark D. The sequence listing filed with the application follows.

SEQUENCE LISTING (5 sequences)

SEQ ID NO: 1 - DNA, 20 bp, Mus musculus
cacctatgccacccttatcc

SEQ ID NO: 2 - DNA, 19 bp, Mus musculus
attgtgggtcaaggggaag

SEQ ID NO: 3 - protein, 21 aa, Artificial
  peptide
MEVGWYRSPFSRVVHLYRNGK

SEQ ID NO: 4 - protein, 17 aa, Artificial
  peptide
ISQAVHAAHAEINEAGR

SEQ ID NO: 5 - protein, 297 aa, Artificial
  PC61scFv
MAKWVTFLLLLFISGSAFSHHHHHHHHHQVVLTQPKSVSASLESTVKLSCKLNSGNIGSYYMHWYQQREGRSPTNLIYRDDKRPDGAPDRFSGSIDISSNSAFLTINNVQTEDEAMYFCHSYDGRMYIFGGGTKLTVLGQPGGGGSGGGGSGGGGSGGGGSQVQLQQSGAELVRPGTSVKLSCKVSGDTITAYYIHFVKQRPGQGLEWIGRIDPEDDSTEYAEKFKNKATITANTSSNTAHLKYSRLTSEDTATYFCTTDNMGATEFVYWGQGTLVTVSSAKGGGSEGGGSEGGGSG